European Patent Application EP 4 420 513 A1, published August 28, 2024. Title: Eustoma root rot-resistance Eustoma plant. Applicant: タキイ種苗株式会社. Application JP. The sequence listing filed with the application follows.

SEQUENCE LISTING (80 sequences)

SEQ ID NO: 1 - DNA, 201 bp, Eustoma grandiflorum
  source 1..201: mol_type = genomic DNA
ttgaccaacacaaggtgtcattctgcaaacaggctttcggtatagcagcagtgaaacactcaaactgtacgtgtccatgggttcaaatttttgatctctttgagcaaatcccaacccgagtactaactgagatatgtcctggggaccgtagcaagatatctaaatgaatgtgcagtctattcctatttttaacttacatat

SEQ ID NO: 2 - DNA, 201 bp, Eustoma grandiflorum
  source 1..201: mol_type = genomic DNA
gctcaaattttttccagctatggaatcagccccagaacaggtttcctttcttttttcttcctgttcaaaagcatccaattttatgcattttggtacctagatttggtgaattttgataaagatttgatctttataattttttattggggcttaggattctgagaaagtcgggtctctaaaggaggtgaagatgaatgaaac

SEQ ID NO: 3 - DNA, 201 bp, Eustoma grandiflorum
  source 1..201: mol_type = genomic DNA
tttacaggagcgtaacgagaggttattttacaagcttctaattgacaatgtggacgaactccttcctgtggtgtacactcccactgttggtgaggcttgcaagaaatatggaagcattttcaagcgtcctcagggtctcttcatcagtttgaaagaaaggttctgtcatttgtttttaatttgtcttaaaacgactactgt

SEQ ID NO: 4 - DNA, 151 bp, Eustoma grandiflorum
  source 1..151: mol_type = genomic DNA
tgaagtttggagagtctctagggctattaaacatgcatcattagtacttcatggtgatttcacatgaaggtgcttgcagaaagaattcacaggaatgcttttttgttgtatatcaaaatattcgtattgaatgtctttttttttttctggc

SEQ ID NO: 5 - DNA, 201 bp, Eustoma grandiflorum
  source 1..201: mol_type = genomic DNA
cacaggtggtaggatggcctccagttcgatcgttccgaaagaattcaatggcaaacaatcctcacaaggctgatgaagaagcagatgcaatgactggaagcagtcgtctttacgtcaaagttagcatggatggtgccccttatctgaggaaagttgatatcaagacatacaacagctacaaggacctgtcctctgcacttg

SEQ ID NO: 6 - DNA, 201 bp, Eustoma grandiflorum
  source 1..201: mol_type = genomic DNA
  variation 101: note = n is T or C
cacaggtggtaggatggcctccagttcgatcgttccgaaagaattcaatggcaaacaatcctcacaaggctgatgaagaagcagatgcaatgactggaagnagtcgtctttacgtcaaagttagcatggatggtgccccttatctgaggaaagttgatatcaagacatacaacagctacaaggacctgtcctctgcacttg

SEQ ID NO: 7 - DNA, 201 bp, Eustoma grandiflorum
  source 1..201: mol_type = genomic DNA
  variation 101: note = n is G or T
ttgaccaacacaaggtgtcattctgcaaacaggctttcggtatagcagcagtgaaacactcaaactgtacgtgtccatgggttcaaatttttgatctcttngagcaaatcccaacccgagtactaactgagatatgtcctggggaccgtagcaagatatctaaatgaatgtgcagtctattcctatttttaacttacatat

SEQ ID NO: 8 - DNA, 101 bp, Eustoma grandiflorum
  source 1..101: mol_type = genomic DNA
  variation 51: note = n is G or A
ttttttcttcctgttcaaaagcatccaattttatgcattttggtacctagntttggtgaattttgataaagatttgatctttataattttttattggggct

SEQ ID NO: 9 - DNA, 101 bp, Eustoma grandiflorum
  source 1..101: mol_type = genomic DNA
  variation 51: note = n is C or A
tggacgaactccttcctgtggtgtacactcccactgttggtgaggcttgcnagaaatatggaagcattttcaagcgtcctcagggtctcttcatcagtttg

SEQ ID NO: 10 - DNA, 151 bp, Eustoma grandiflorum
  source 1..151: mol_type = genomic DNA
  variation 76: note = n is A or G
tgaagtttggagagtctctagggctattaaacatgcatcattagtacttcatggtgatttcacatgaaggtgcttncagaaagaattcacaggaatgcttttttgttgtatatcaaaatattcgtattgaatgtctttttttttttctggc

SEQ ID NO: 11 - DNA, 101 bp, Eustoma grandiflorum
  source 1..101: mol_type = genomic DNA
  variation 51: note = n is T or G
aaaaagtgaggatttttttttggggttgtgtttgacaaagggttcttaacngcaagaaaatgtattttctgttgctttgacagaattattttccgacaatt

SEQ ID NO: 12 - DNA, 101 bp, Eustoma grandiflorum
  source 1..101: mol_type = genomic DNA
  variation 51: note = n is A or T
agacgccgttgtctgtctccgcttgacatgcccaaaccatctcagtttccnatttcttatcttatccgctatactaatcacccctagccttttccgaaata

SEQ ID NO: 13 - DNA, 101 bp, Eustoma grandiflorum
  source 1..101: mol_type = genomic DNA
  variation 51: note = n is T or A
tttctgcagtatgtgaaaatgggtatccgaaatggacgttctagataaaanattttacattggcatgaaaaagcaaaagtaagcaaaacataattattcat

SEQ ID NO: 14 - DNA, 101 bp, Eustoma grandiflorum; identical to SEQ ID NO: 8
  source 1..101: mol_type = genomic DNA
  variation 51: note = n is G or A

SEQ ID NO: 15 - DNA, 101 bp, Eustoma grandiflorum
  source 1..101: mol_type = genomic DNA
  variation 51: note = n is T or G
atcaaaaatcagataaaaaagggattagattttaatttttaaacatgtagntttcaattttagtttttaatcttattaattaataatattgttgttaagat

SEQ ID NO: 16 - DNA, 101 bp, Eustoma grandiflorum
  source 1..101: mol_type = genomic DNA
  variation 51: note = n is C or A
tattccgttgactggtgttgactaacagacgattaattatggtttatcacnctcaattaacaccaaactctatttgtctgatctgacggaataacaatacc

SEQ ID NO: 17 - DNA, 101 bp, Eustoma grandiflorum
  source 1..101: mol_type = genomic DNA
  variation 51: note = n is T or C
gttgttgttgttctattgtgtctctagttactctttacttattctcaaagnaacataaaacctcccagtaaccaaattgtcatttagatcatcatcatcat

SEQ ID NO: 18 - DNA, 101 bp, Eustoma grandiflorum
  source 1..101: mol_type = genomic DNA
  variation 51: note = n is G or A
atgtcacttctagaactgatttgtgccttttatttgtgtggtttttggttngatcatctgtatgagtacgcaatattttggtttaatgttgatcttaatca

SEQ ID NO: 19 - DNA, 101 bp, Eustoma grandiflorum; identical to SEQ ID NO: 9
  source 1..101: mol_type = genomic DNA
  variation 51: note = n is C or A

SEQ ID NO: 20 - DNA, 101 bp, Eustoma grandiflorum
  source 1..101: mol_type = genomic DNA
  variation 51: note = n is T or C
ttctgaagttgtttatgaatggatctgagagatcatactggttgttcaatnaattgaaggcagctgtggttgattgctgtggtcaatgaaacatggaaaaa

SEQ ID NO: 21 - DNA, 101 bp, Eustoma grandiflorum
  source 1..101: mol_type = genomic DNA
  variation 51: note = n is G or T
tggttcagaagtttgcatgaaatgacactaactgattgaatttaaacagtntagcagcttgttaggacagtgtgttcaaatttttcataagggtacctctc

SEQ ID NO: 22 - DNA, 101 bp, Eustoma grandiflorum
  source 1..101: mol_type = genomic DNA
  variation 51: note = n is G or T
tttgttgcagataattaccatctgaagaggatgcagaaacaagaataatcngtgtaaaatcccaagaatcatattcaggaacctcgttcaaccaaataaca

SEQ ID NO: 23 - DNA, 101 bp, Eustoma grandiflorum
  source 1..101: mol_type = genomic DNA
  variation 51: note = n is C or T
tcagatatacgcagtcatacccatgtgttagaaacatacaaaggttgttcncgatgaccataatgaaaattgtgtctgtcgatctgtagcgccccgctccc

SEQ ID NO: 24 - DNA, 101 bp, Eustoma grandiflorum
  source 1..101: mol_type = genomic DNA
  variation 51: note = n is C or T
gaatacaatttttacaatattcagcctccaaattccatccttccattttanaattgttcttacatattccacaatgtgtgatcttctaaatgttctttaaa

SEQ ID NO: 25 - DNA, 101 bp, Eustoma grandiflorum
  source 1..101: mol_type = genomic DNA
  variation 51: note = n is A or T
gtgcagaagaaaaaaaaagaagaagaagaagaagctgcgaagagaatatgnctggccaaaatattttctcttctattgaaaactgtttttagaaaagactc

SEQ ID NO: 26 - DNA, 101 bp, Eustoma grandiflorum
  source 1..101: mol_type = genomic DNA
  variation 51: note = n is T or G
gctaaaacactttcttcaaaactcttcactcttcgtcttgataccattttntaaaaatgtttttcatctcttggctgtgaagagtcattgcctttggcagg

SEQ ID NO: 27 - DNA, 101 bp, Eustoma grandiflorum
  source 1..101: mol_type = genomic DNA
  variation 51: note = n is G or C
actactttaaaactttgtttccaacaggcagtgaagagccttagtcttgtnctgaaatcttctaaccttcaaatctttttcaatagactgtgaagggcctt

SEQ ID NO: 28 - DNA, 101 bp, Eustoma grandiflorum
  source 1..101: mol_type = genomic DNA
  variation 51: note = n is C or T
tgaactcaacctgatgtcattaaaggcttctttgttttcaactcatactgntcaaacatacaaacttttctaaaactatgccattgaatctcctaatatat

SEQ ID NO: 29 - DNA, 101 bp, Eustoma grandiflorum
  source 1..101: mol_type = genomic DNA
  variation 51: note = n is G or A
acacaacaggtgcagtgctcaactcagccaaactactataagtattgaccnagctgagctgaccacaagtgtacaactacgtactgctgataccctttcat

SEQ ID NO: 30 - DNA, 101 bp, Eustoma grandiflorum
  source 1..101: mol_type = genomic DNA
  variation 51: note = n is A or G
catgtggaaaatggtcaatgattgtgagctgattgacctggggtactctgntccagcattcacttggaccaatctcagggatgacgaggacaatatcatgg

SEQ ID NO: 31 - DNA, 101 bp, Eustoma grandiflorum
  source 1..101: mol_type = genomic DNA
  variation 51: note = n is G or A
tacactacacaaatcacaactccctgccccccacacatgatctcattctcnccacttacagagggggacctcacgagcctgaatagggaggtgatccctca

SEQ ID NO: 32 - DNA, 101 bp, Eustoma grandiflorum
  source 1..101: mol_type = genomic DNA
  variation 7: note = n is C or T
  variation 51: note = n is G or A
ccattcngccaaaacatatcttaattgccaggattttgaaggaaacaggcnaaattttgaaggttctggagaaggaaaacgaaaggaaagaggtggaatgg

SEQ ID NO: 33 - DNA, 93 bp, Eustoma grandiflorum
  source 1..93: mol_type = genomic DNA
  variation 4: note = n is T or A
  variation 7: note = n is T or C
  variation 9: note = n is C or G
  variation 33: note = n is C or T
  variation 42: note = n is A or G
  variation 43: note = n is A or G
attnacntnatccgttacagtcaattatataanctttacagnnacgcaagttgcttatggttcatattagccactcgggtcctaatatacagt

SEQ ID NO: 34 - DNA, 101 bp, Eustoma grandiflorum
  source 1..101: mol_type = genomic DNA
  variation 51: note = n is T or G
ccattgggatggactgctagggagataactttgttctgcttgaatgtgctntaaggtcaattggtagaggcaaatgtattctgctgctttaggtaaatacc

SEQ ID NO: 35 - DNA, 101 bp, Eustoma grandiflorum
  source 1..101: mol_type = genomic DNA
  variation 45: note = n is C or T
  variation 51: note = n is A or G
gcaaatgtattctgctgctttaggtaaataccgtatcctgccttnattttntatcttaaaagttgtttgctttaaagttatcaatcattattactccataa

SEQ ID NO: 36 - DNA, 101 bp, Eustoma grandiflorum
  source 1..101: mol_type = genomic DNA
  variation 51: note = n is A or T
taaaagttgtttgctttaaagttatcaatcattattactccataaggaaangcaattatttcttaggcgaaatgcaactattactagtagctttttggtgg

SEQ ID NO: 37 - DNA, 101 bp, Eustoma grandiflorum
  source 1..101: mol_type = genomic DNA
  variation 51: note = n is T or C
caattcttcctaatctcgttttctactcttttttcgcttcacatcattttntctcatcatctaacacctgttgttactagggggaagattccagatacata

SEQ ID NO: 38 - DNA, 101 bp, Eustoma grandiflorum
  source 1..101: mol_type = genomic DNA
  variation 51: note = n is A or G
tgataccggtatgtttcgaaggtggagtgaggatgctgattacctgctagnatccgggtttcagcaaataaatagtttcttacctgcggttgcgagtatca

SEQ ID NO: 39 - DNA, 101 bp, Eustoma grandiflorum
  source 1..101: mol_type = genomic DNA
  variation 51: note = n is T or A
acaatcattttggcgatattgaacgttgcagtttataaattgaagcaaatntgcaaattcacattctggcaggagaaagatatgcaatcagctccagataa

SEQ ID NO: 40 - DNA, 101 bp, Eustoma grandiflorum
  source 1..101: mol_type = genomic DNA
  variation 51: note = n is T or C
ttcggtaaagtatacagaggttttctttacgggcgtccagaaattcttgcnataaagcgattgaagcccgactccaaacaaggggcacatgaattttggcg

SEQ ID NO: 41 - DNA, 101 bp, Eustoma grandiflorum
  source 1..101: mol_type = genomic DNA
  variation 51: note = n is A or G
  variation 97: note = n is G or C
gagaattttgttgctaagatttcagattttgggctatcaaaactgggtagnacaggggaaatcctgagccaacttagcacaaaaattaaaggcacanttgg

SEQ ID NO: 42 - DNA, 101 bp, Eustoma grandiflorum
  source 1..101: mol_type = genomic DNA
  variation 51: note = n is T or C
  variation 81: note = n is T or C
caacttagcacaaaaattaaaggcacagttggttatctggatcctgattancttatgactcataaaccttcaacaaaaagngatatatatgcatttggcat

SEQ ID NO: 43 - DNA, 101 bp, Eustoma grandiflorum
  source 1..101: mol_type = genomic DNA
  variation 49: note = n is A or G
  variation 51: note = n is C or T
cgtatcttctctctaaaagaaattaaatcagccaccaaaaactttagcnanagtttccttattggccagggaggatacggtaaagtgtacaaaggtttcat

SEQ ID NO: 44 - DNA, 101 bp, Eustoma grandiflorum
  source 1..101: mol_type = genomic DNA
  variation 39: note = n is A or G
  variation 51: note = n is C or G
tcaagagatggagctcttactccacgcagagtgcttcanatttccacacanaagttcaattactacccaagctccagttcattcatctcgtatcttttgtg

SEQ ID NO: 45 - DNA, 101 bp, Eustoma grandiflorum
  source 1..101: mol_type = genomic DNA
  variation 51: note = n is G or A
  variation 92: note = n is A or T
aaggttcacttgatactcatctctatggaggcactgtaaacagaaagaacnttacgtctctcacttgggagcaaagactcataatctgcacnggtgctgct

SEQ ID NO: 46 - DNA, 101 bp, Eustoma grandiflorum
  source 1..101: mol_type = genomic DNA
  variation 51: note = n is G or A
  variation 63: note = n is T or C
agcaagagaaaatgcagctgccaccctttttagcttatcaatcttcgatgngaacaaggtagntataggtgcagctggggccataccgcccctcgttgatt

SEQ ID NO: 47 - DNA, 101 bp, Eustoma grandiflorum
  source 1..101: mol_type = genomic DNA
  variation 51: note = n is A or T
gatcattgttcaaggagatgaccaacaagtagaccagatgagaagagagcnccagcttactgaataaggaatgatttatgttaaaggcatgtttgagagat

SEQ ID NO: 48 - DNA, 101 bp, Eustoma grandiflorum
  source 1..101: mol_type = genomic DNA
  variation 51: note = n is G or A
ggccttcagaaacagagaatcagtgctgctattaggcatcggtttggatcnaaaagcagaggcagccatgcagatattatgttaatggtagctatacgttg

SEQ ID NO: 49 - DNA, 101 bp, Eustoma grandiflorum
  source 1..101: mol_type = genomic DNA
  variation 51: note = n is G or T
gctgcatcgagatttcaagaatcaagatcaaagcacatcaatccccaattnccctaacgttctgagcaattcttcaaaataaaagtactccccagtcaaca

SEQ ID NO: 50 - DNA, 85 bp, Eustoma grandiflorum
  source 1..85: mol_type = genomic DNA
  variation 51: note = n is A or G
atcccatcgcttttagaagaaaacaaagtccaagcccattcataaataacnatttaatgtattttgaaacttgttttagatcact

SEQ ID NO: 51 - DNA, 101 bp, Eustoma grandiflorum
  source 1..101: mol_type = genomic DNA
  variation 51: note = n is T or C
ttaatgtattttgaaacttgttttagatcacttcgccaacacgaaacccanattccagcccacttaataaaagataaagcccacaacatttgggcctttta

SEQ ID NO: 52 - DNA, 91 bp, Eustoma grandiflorum
  source 1..91: mol_type = genomic DNA
  variation 51: note = n is T or C
gtcgtctgattggacatgaaaaaaattcggccataaattagacctgccaanaaaacacccttaatgataattactttcgtcaagtctcata

SEQ ID NO: 53 - DNA, 101 bp, Eustoma grandiflorum
  source 1..101: mol_type = genomic DNA
  variation 51: note = n is T or A
aaaagttcatgcttaaaagaatttataacctatgaaaccacacgaactttnagtacattagggcaaatatttgctttgcaggcaccccctccatcattgca

SEQ ID NO: 54 - DNA, 101 bp, Eustoma grandiflorum
  source 1..101: mol_type = genomic DNA
  variation 51: note = n is T or C
attataaaaacgaataatcgtacaaaaattaaagttgtctatttaattatnaacttttgtaccgcactttcaattgctttacgttgaaagatggaaaaggt

SEQ ID NO: 55 - DNA, 101 bp, Eustoma grandiflorum
  source 1..101: mol_type = genomic DNA
  variation 51: note = n is C or T
cactgcttagctaaatgccagtttgctgggggacaccttgtgtgggtcacngcataagtcatcacccaacctagaaggccgctgagctcctgatttatatc

SEQ ID NO: 56 - DNA, 101 bp, Eustoma grandiflorum
  source 1..101: mol_type = genomic DNA
  variation 51: note = n is G or A
aacactattgtttatttttttttacataggtatactaagataagatttganctctaatttttaccaatatggcgttttaaaacactactctttgttttttt

SEQ ID NO: 57 - DNA, 102 bp, Eustoma grandiflorum
  source 1..102: mol_type = genomic DNA
  variation 8: note = n is deletion or A
  variation 52: note = n is G or A
  variation 60: note = n is T or deletion
acttaaancagtcttagtaaacatgcatctatcaataataaattccattagnaggtgttnctaagttttgccttaaaagtaaaatctactttggagggcaat

SEQ ID NO: 58 - DNA, 101 bp, Eustoma grandiflorum
  source 1..101: mol_type = genomic DNA
  variation 8: note = n is T or deletion
  variation 51: note = n is A or G
aggtgttnctaagttttgccttaaaagtaaaatctactttggagggcaatngtgtcctcaaaagattctaagaaggagtgatggactttttggtggggaaa

SEQ ID NO: 59 - DNA, 101 bp, Eustoma grandiflorum
  source 1..101: mol_type = genomic DNA
  variation 51: note = n is A or C
  variation 69: note = n is T or G
  variation 84: note = n is G or C
  variation 85: note = n is G or A
  variation 89: note = n is T or G
  variation 95: note = n is A or G
  variation 98: note = n is C or T
tcaaaagattctaagaaggagtgatggactttttggtggggaaattacccnatcggaaaacaaacgtgngtttctaacacatgnntatnattacntanatc

SEQ ID NO: 60 - DNA, 101 bp, Eustoma grandiflorum
  source 1..101: mol_type = genomic DNA
  variation 51: note = n is C or A
ttattctttattttgtgcaagaggttgtttccacggctcgaactcctaacntcaaagtcacaaaacagcaaccgtaccagttgctacaagaaccgtcgttc

SEQ ID NO: 61 - DNA, 101 bp, Eustoma grandiflorum
  source 1..101: mol_type = genomic DNA
  variation 51: note = n is A or T
tataggggcatctagagtacacttaggcgtttagatgctctctagactttntgttgactttgcacttttttgtacttttgtgtttatgttttggtctttaa

SEQ ID NO: 62 - DNA, 101 bp, Eustoma grandiflorum
  source 1..101: mol_type = genomic DNA
  variation 51: note = n is A or G
tcttatcccgcatttcgccccttggttactttcaatgaagagacacccatncgaacaaatttttctttttcgtttctcagtctggaagcgatgtgccaatt

SEQ ID NO: 63 - DNA, 101 bp, Eustoma grandiflorum
  source 1..101: mol_type = genomic DNA
  variation 51: note = n is T or G
ttctcagtctggaagcgatgtgccaatttttttttcaattaattgataaantgctatctaattaaatcaaatatatatatatgaagaaaagaaaatattta

SEQ ID NO: 64 - DNA, 101 bp, Eustoma grandiflorum
  source 1..101: mol_type = genomic DNA
  variation 51: note = n is C or A
agttcggttcgcttaacacctctaacaatgttatattaaaagttgtaaaantacaatattacagcaagcaccagatgggatctactaccaaccttagatat

SEQ ID NO: 65 - DNA, 101 bp, Eustoma grandiflorum
  source 1..101: mol_type = genomic DNA
  variation 51: note = n is T or C
acataaaagtgaaaagtgcaggttggaaggctaggagcaggatcagattangcagcatttctacaacatgttggtgttccagctgttgacatggcttttgg

SEQ ID NO: 66 - DNA, 101 bp, Eustoma grandiflorum
  source 1..101: mol_type = genomic DNA
  variation 51: note = n is T or G
cagctgttgacatggcttttggagaaggtaatagaacagacttgtctacanatattcctttttcatacggcataccatgaaaagtgcattgtagtacaaca

SEQ ID NO: 67 - DNA, 101 bp, Eustoma grandiflorum
  source 1..101: mol_type = genomic DNA
  variation 51: note = n is T or C
cacttgtccaccatagactgcttccttcctttctgtgaaatccttttaccncagcacagctacagggcagtcgcaagggagaagaagaaacaaaaaaagtc

SEQ ID NO: 68 - DNA, 101 bp, Eustoma grandiflorum
  source 1..101: mol_type = genomic DNA
  variation 51: note = n is A or C
aaactaatattagtcatagatcgagtaaaacagaatatctaactacatagnacataatcaactaggtaaacagctactagcgactgtaattggcaacttcg

SEQ ID NO: 69 - DNA, 101 bp, Eustoma grandiflorum
  source 1..101: mol_type = genomic DNA
  variation 51: note = n is T or C
ttttcctttgagttttccttatggaagagttatgatcattatctttgtgtntgaaacattcacgattagcatttaaactagatgacccatagtctctgtgg

SEQ ID NO: 70 - DNA, 101 bp, Eustoma grandiflorum
  source 1..101: mol_type = genomic DNA
  variation 51: note = n is C or T
aatgcagattaaggtacagcttgacttgagctgttcaggttttagtaaaantttatcctgtttagattttgataaaggaaactggtcaaggcactacaagg

SEQ ID NO: 71 - DNA, 101 bp, Eustoma grandiflorum
  source 1..101: mol_type = genomic DNA
  variation 51: note = n is G or A
gtcaaggcactacaaggcagcaaaggctgggtatcagcttggagatatgangcagggaaagtgagagaggtgaatgacagactaatgatggcagaaagagc

SEQ ID NO: 72 - DNA, 101 bp, Eustoma grandiflorum
  source 1..101: mol_type = genomic DNA
atgtcacttctagaactgatttgtgccttttatttgtgtggtttttggttagatcatctgtatgagtacgcaatattttggtttaatgttgatcttaatca

SEQ ID NO: 73 - DNA, 101 bp, Eustoma grandiflorum
  source 1..101: mol_type = genomic DNA
tttgttgcagataattaccatctgaagaggatgcagaaacaagaataatctgtgtaaaatcccaagaatcatattcaggaacctcgttcaaccaaataaca

SEQ ID NO: 74 - DNA, 101 bp, Eustoma grandiflorum
  source 1..101: mol_type = genomic DNA
gaatacaatttttacaatattcagcctccaaattccatccttccattttataattgttcttacatattccacaatgtgtgatcttctaaatgttctttaaa

SEQ ID NO: 75 - DNA, 101 bp, Eustoma grandiflorum
  source 1..101: mol_type = genomic DNA
acacaacaggtgcagtgctcaactcagccaaactactataagtattgaccaagctgagctgaccacaagtgtacaactacgtactgctgataccctttcat

SEQ ID NO: 76 - DNA, 101 bp, Eustoma grandiflorum
  source 1..101: mol_type = genomic DNA
tgataccggtatgtttcgaaggtggagtgaggatgctgattacctgctaggatccgggtttcagcaaataaatagtttcttacctgcggttgcgagtatca

SEQ ID NO: 77 - DNA, 101 bp, Eustoma grandiflorum
  source 1..101: mol_type = genomic DNA
gctgcatcgagatttcaagaatcaagatcaaagcacatcaatccccaatttccctaacgttctgagcaattcttcaaaataaaagtactccccagtcaaca

SEQ ID NO: 78 - DNA, 101 bp, Eustoma grandiflorum
  source 1..101: mol_type = genomic DNA
ttattctttattttgtgcaagaggttgtttccacggctcgaactcctaacatcaaagtcacaaaacagcaaccgtaccagttgctacaagaaccgtcgttc

SEQ ID NO: 79 - DNA, 101 bp, Eustoma grandiflorum
  source 1..101: mol_type = genomic DNA
ttttttcttcctgttcaaaagcatccaattttatgcattttggtacctagatttggtgaattttgataaagatttgatctttataattttttattggggct

SEQ ID NO: 80 - DNA, 101 bp, Eustoma grandiflorum
  source 1..101: mol_type = genomic DNA
tggacgaactccttcctgtggtgtacactcccactgttggtgaggcttgcaagaaatatggaagcattttcaagcgtcctcagggtctcttcatcagtttg